European Patent Application EP 4 414 365 A1, published August 14, 2024. Title: PYRIDAZINONES AND METHODS OF USE THEREOF. Applicant: GOLDFINCH BIO, INC. Application EP, filed September 18, 2019. The sequence listing filed with the application follows.

SEQUENCE LISTING (2 sequences)

SEQ ID NO: 1 - DNA, 8574 bp, synthetic construct
  misc_feature 1..8574: note = Description of Artificial Sequence: Synthetic polynucleotide
  source 1..8574: mol_type = other DNA
gacggatcgggagatctcccgatcccctatggtgcactctcagtacaatctgctctgatgccgcatagttaagccagtatctgctccctgcttgtgtgttggaggtcgctgagtagtgcgcgagcaaaatttaagctacaacaaggcaaggcttgaccgacaattgcatgaagaatctgcttagggttaggcgttttgcgctgcttcgcgatgtacgggccagatatacgcgttgacattgattattgactagttattaatagtaatcaattacggggtcattagttcatagcccatatatggagttccgcgttacataacttacggtaaatggcccgcctggctgaccgcccaacgacccccgcccattgacgtcaataatgacgtatgttcccatagtaacgccaatagggactttccattgacgtcaatgggtggagtatttacggtaaactgcccacttggcagtacatcaagtgtatcatatgccaagtacgccccctattgacgtcaatgacggtaaatggcccgcctggcattatgcccagtacatgaccttatgggactttcctacttggcagtacatctacgtattagtcatcgctattaccatggtgatgcggttttggcagtacatcaatgggcgtggatagcggtttgactcacggggatttccaagtctccaccccattgacgtcaatgggagtttgttttggcaccaaaatcaacgggactttccaaaatgtcgtaacaactccgccccattgacgcaaatgggcggtaggcgtgtacggtgggaggtctatataagcagagctctccctatcagtgatagagatctccctatcagtgatagagatcgtcgacgagctcgtttagtgaaccgtcagatcgcctggagacgccatccacgctgttttgacctccatagaagacaccgggaccgatccagcctccggactctagcgtttaaacttaagcttggtaccgagctcggatccgccaccatggcccagttctactataagagaaacgtgaatgccccttaccgcgacagaatccccctgagaatcgtgagggcagagtccgagctgagcccatccgagaaggcctacctgaacgccgtggagaagggcgactatgccagcgtgaagaagtccctggaggaggccgagatctactttaagatcaacatcaattgcatcgatcctctgggcagaaccgccctgctgatcgccatcgagaacgagaatctggagctgatcgagctgctgctgagcttcaacgtgtatgtgggcgatgccctgctgcacgccatcaggaaggaggtggtgggagcagtggagctgctgctgaatcacaagaagccaagcggagagaagcaggtgccacctatcctgctggacaagcagttctccgagtttaccccagatatcacacccatcatcctggccgcccacaccaacaattacgagatcatcaagctgctggtgcagaagggcgtgtccgtgcctcgcccacacgaggtgcggtgcaactgcgtggagtgcgtgagctcctctgacgtggattctctgaggcacagccggagccggctgaacatctataaggccctggcctccccatctctgatcgccctgagctccgaggaccccttcctgaccgcctttcagctgtcttgggagctgcaggagctgagcaaggtggagaacgagtttaagagcgagtacgaggagctgtccagacagtgcaagcagttcgccaaggacctgctggatcagacacgctctagccgggagctggagatcatcctgaactatagggacgataattctctgatcgaggagcagagcggaaacgacctggcacgcctgaagctggccatcaagtaccggcagaaggagttcgtggcccagcctaattgtcagcagctgctggcctcccgctggtatgatgagtttccaggatggcggagaaggcactgggcagtgaagatggtgacctgcttcatcatcggcctgctgttccccgtgttcagcgtgtgctacctgatcgcccctaagtctccactgggcctgtttatccggaagcctttcatcaagtttatctgccacaccgccagctatctgacattcctgtttctgctgctgctggcctcccagcacatcgacagatctgatctgaacaggcagggcccaccccctaccatcgtggagtggatgatcctgccatgggtgctgggcttcatctggggcgagatcaagcagatgtgggacggcggcctgcaggactacatccacgattggtggaacctgatggattttgtgatgaattccctgtacctggccacaatctctctgaagatcgtggccttcgtgaagtatagcgccctgaatcccagagagtcctgggacatgtggcaccctaccctggtggcagaggccctgttcgcaatcgccaacatcttttcctctctgcgcctgatcagcctgtttacagccaattcccacctgggaccactgcagatctccctgggacggatgctgctggatatcctgaagttcctgtttatctactgcctggtgctgctggccttcgccaacggcctgaatcagctgtacttctactatgaggagaccaagggcctgacatgcaagggcatccgctgtgagaagcagaacaatgccttcagcaccctgttcgagacactgcagtctctgttctggagcatctttggcctgatcaacctgtacgtgaccaatgtgaaggcccagcacgagttcacagagtttgtgggcgccaccatgttcggcacatacaacgtgatctctctggtggtgctgctgaatatgctgatcgccatgatgaacaatagctatcagctgatcgccgaccacgccgatatcgagtggaagttcgcccggaccaagctgtggatgtcctactttgaggagggcggcaccctgcccacacctttcaacgtgatcccatcccccaagtctctgtggtatctgatcaagtggatctggacacacctgtgcaagaagaagatgcgccggaagcctgagagctttggcaccatcggcgtgcgcacacagcacagaagggcagcagacaacctgcgccggcaccaccagtaccaggaagtgatgcgcaatctggtgaagcggtatgtggccgccatgatcagggacgcaaagaccgaggagggactgacagaggagaacttcaaggagctgaagcaggatatcagctccttcagatttgaggtgctgggcctgctgaggggcagcaagctgtccaccatccagtccgccaacgcctctaaggagtctagcaattctgccgacagcgatgagaagagcgactccgagggcaactctaaggataagaagaagaacttcagcctgtttgacctgaccacactgatccacccacgcagcgccgcaatcgcatccgagcggcacaacatctccaatggctctgccctggtggtgcaggagccaccaagagagaagcagaggaaggtgaactttgtgacagatatcaagaatttcggcctgtttcacagaaggagcaagcagaacgccgccgagcagaacgccaatcagatcttctctgtgagcgaggaggtggcaagacagcaggcagcaggaccactggagaggaatatccagctggagagccggggactggcaagcaggggcgacctgtccatcccaggactgtctgagcagtgcgtgctggtggaccacagggagcggaacaccgatacactgggactgcaagtgggcaagcgggtgtgccctttcaagagcgagaaggtcgtggtggaggacaccgtgcccatcatccctaaggagaagcacgccaaggaggaggattcctctatcgactacgatctgaatctgccagacaccgtgacacacgaggattatgtgaccacaaggctgtgagcggccgctctagagggcccgtttaaacccgctgatcagcctcgactgtgccttctagttgccagccatctgttgtttgcccctcccccgtgccttccttgaccctggaaggtgccactcccactgtcctttcctaataaaatgaggaaattgcatcgcattgtctgagtaggtgtcattctattctggggggtggggtggggcaggacagcaagggggaggattgggaagacaatagcaggcatgctggggatgcggtgggctctatggcttctgaggcggaaagaaccagctggggctctagggggtatccccacgcgccctgtagcggcgcattaagcgcggcgggtgtggtggttacgcgcagcgtgaccgctacacttgccagcgccctagcgcccgctcctttcgctttcttcccttcctttctcgccacgttcgccggctttccccgtcaagctctaaatcgggggctccctttagggttccgatttagtgctttacggcacctcgaccccaaaaaacttgattagggtgatggttcacgtagtgggccatcgccctgatagacggtttttcgccctttgacgttggagtccacgttctttaatagtggactcttgttccaaactggaacaacactcaaccctatctcggtctattcttttgatttataagggattttgccgatttcggcctattggttaaaaaatgagctgatttaacaaaaatttaacgcgaattaattctgtggaatgtgtgtcagttagggtgtggaaagtccccaggctccccagcaggcagaagtatgcaaagcatgcatctcaattagtcagcaaccaggtgtggaaagtccccaggctccccagcaggcagaagtatgcaaagcatgcatctcaattagtcagcaaccatagtcccgcccctaactccgcccatcccgcccctaactccgcccagttccgcccattctccgccccatggctgactaattttttttatttatgcagaggccgaggccgcctctgcctctgagctattccagaagtagtgaggaggcttttttggaggcctaggcttttgcaaaaagctcccgggagcttgtatatccattttcggatctgatcagcacgtgatgaaaaagcctgaactcaccgcgacgtctgtcgagaagtttctgatcgaaaagttcgacagcgtctccgacctgatgcagctctcggagggcgaagaatctcgtgctttcagcttcgatgtaggagggcgtggatatgtcctgcgggtaaatagctgcgccgatggtttctacaaagatcgttatgtttatcggcactttgcatcggccgcgctcccgattccggaagtgcttgacattggggaattcagcgagagcctgacctattgcatctcccgccgtgcacagggtgtcacgttgcaagacctgcctgaaaccgaactgcccgctgttctgcagccggtcgcggaggccatggatgcgatcgctgcggccgatcttagccagacgagcgggttcggcccattcggaccgcaaggaatcggtcaatacactacatggcgtgatttcatatgcgcgattgctgatccccatgtgtatcactggcaaactgtgatggacgacaccgtcagtgcgtccgtcgcgcaggctctcgatgagctgatgctttgggccgaggactgccccgaagtccggcacctcgtgcacgcggatttcggctccaacaatgtcctgacggacaatggccgcataacagcggtcattgactggagcgaggcgatgttcggggattcccaatacgaggtcgccaacatcttcttctggaggccgtggttggcttgtatggagcagcagacgcgctacttcgagcggaggcatccggagcttgcaggatcgccgcggctccgggcgtatatgctccgcattggtcttgaccaactctatcagagcttggttgacggcaatttcgatgatgcagcttgggcgcagggtcgatgcgacgcaatcgtccgatccggagccgggactgtcgggcgtacacaaatcgcccgcagaagcgcggccgtctggaccgatggctgtgtagaagtactcgccgatagtggaaaccgacgccccagcactcgtccgagggcaaaggaatagcacgtgctacgagatttcgattccaccgccgccttctatgaaaggttgggcttcggaatcgttttccgggacgccggctggatgatcctccagcgcggggatctcatgctggagttcttcgcccaccccaacttgtttattgcagcttataatggttacaaataaagcaatagcatcacaaatttcacaaataaagcatttttttcactgcattctagttgtggtttgtccaaactcatcaatgtatcttatcatgtctgtataccgtcgacctctagctagagcttggcgtaatcatggtcatagctgtttcctgtgtgaaattgttatccgctcacaattccacacaacatacgagccggaagcataaagtgtaaagcctggggtgcctaatgagtgagctaactcacattaattgcgttgcgctcactgcccgctttccagtcgggaaacctgtcgtgccagctgcattaatgaatcggccaacgcgcggggagaggcggtttgcgtattgggcgctcttccgcttcctcgctcactgactcgctgcgctcggtcgttcggctgcggcgagcggtatcagctcactcaaaggcggtaatacggttatccacagaatcaggggataacgcaggaaagaacatgtgagcaaaaggccagcaaaaggccaggaaccgtaaaaaggccgcgttgctggcgtttttccataggctccgcccccctgacgagcatcacaaaaatcgacgctcaagtcagaggtggcgaaacccgacaggactataaagataccaggcgtttccccctggaagctccctcgtgcgctctcctgttccgaccctgccgcttaccggatacctgtccgcctttctcccttcgggaagcgtggcgctttctcatagctcacgctgtaggtatctcagttcggtgtaggtcgttcgctccaagctgggctgtgtgcacgaaccccccgttcagcccgaccgctgcgccttatccggtaactatcgtcttgagtccaacccggtaagacacgacttatcgccactggcagcagccactggtaacaggattagcagagcgaggtatgtaggcggtgctacagagttcttgaagtggtggcctaactacggctacactagaagaacagtatttggtatctgcgctctgctgaagccagttaccttcggaaaaagagttggtagctcttgatccggcaaacaaaccaccgctggtagcggttggttttttgtttgcaagcagcagattacgcgcagaaaaaaaggatctcaagaagatcctttgatcttttctacggggtctgacgctcagtggaacgaaaactcacgttaagggattttggtcatgagattatcaaaaaggatcttcacctagatccttttaaattaaaaatgaagttttaaatcaatctaaagtatatatgagtaaacttggtctgacagttaccaatgcttaatcagtgaggcacctatctcagcgatctgtctatttcgttcatccatagttgcctgactccccgtcgtgtagataactacgatacgggagggcttaccatctggccccagtgctgcaatgataccgcgagacccacgctcaccggctccagatttatcagcaataaaccagccagccggaagggccgagcgcagaagtggtcctgcaactttatccgcctccatccagtctattaattgttgccgggaagctagagtaagtagttcgccagttaatagtttgcgcaacgttgttgccattgctacaggcatcgtggtgtcacgctcgtcgtttggtatggcttcattcagctccggttcccaacgatcaaggcgagttacatgatcccccatgttgtgcaaaaaagcggttagctccttcggtcctccgatcgttgtcagaagtaagttggccgcagtgttatcactcatggttatggcagcactgcataattctcttactgtcatgccatccgtaagatgcttttctgtgactggtgagtactcaaccaagtcattctgagaatagtgtatgcggcgaccgagttgctcttgcccggcgtcaatacgggataataccgcgccacatagcagaactttaaaagtgctcatcattggaaaacgttcttcggggcgaaaactctcaaggatcttaccgctgttgagatccagttcgatgtaacccactcgtgcacccaactgatcttcagcatcttttactttcaccagcgtttctgggtgagcaaaaacaggaaggcaaaatgccgcaaaaaagggaataagggcgacacggaaatgttgaatactcatactcttcctttttcaatattattgaagcatttatcagggttattgtctcatgagcggatacatatttgaatgtatttagaaaaataaacaaataggggttccgcgcacatttccccgaaaagtgccacctgacgtc

SEQ ID NO: 2 - DNA, 8541 bp, synthetic construct
  misc_feature 1..8541: note = Description of Artificial Sequence: Synthetic polynucleotide
  source 1..8541: mol_type = other DNA
gacggatcgggagatctcccgatcccctatggtgcactctcagtacaatctgctctgatgccgcatagttaagccagtatctgctccctgcttgtgtgttggaggtcgctgagtagtgcgcgagcaaaatttaagctacaacaaggcaaggcttgaccgacaattgcatgaagaatctgcttagggttaggcgttttgcgctgcttcgcgatgtacgggccagatatacgcgttgacattgattattgactagttattaatagtaatcaattacggggtcattagttcatagcccatatatggagttccgcgttacataacttacggtaaatggcccgcctggctgaccgcccaacgacccccgcccattgacgtcaataatgacgtatgttcccatagtaacgccaatagggactttccattgacgtcaatgggtggagtatttacggtaaactgcccacttggcagtacatcaagtgtatcatatgccaagtacgccccctattgacgtcaatgacggtaaatggcccgcctggcattatgcccagtacatgaccttatgggactttcctacttggcagtacatctacgtattagtcatcgctattaccatggtgatgcggttttggcagtacatcaatgggcgtggatagcggtttgactcacggggatttccaagtctccaccccattgacgtcaatgggagtttgttttggcaccaaaatcaacgggactttccaaaatgtcgtaacaactccgccccattgacgcaaatgggcggtaggcgtgtacggtgggaggtctatataagcagagctctccctatcagtgatagagatctccctatcagtgatagagatcgtcgacgagctcgtttagtgaaccgtcagatcgcctggagacgccatccacgctgttttgacctccatagaagacaccgggaccgatccagcctccggactctagcgtttaaacttaagcccaagctggctagaccgccatggcccaactgtactacaaaaaggtcaactactcaccgtacagagaccgcatccccctgcaaattgtgagggctgagacagagctctctgcagaggagaaggccttcctcaatgctgtggagaagggggactatgccactgtgaagcaggcccttcaggaggctgagatctactataatgttaacatcaactgcatggaccccttgggccggagtgccctgctcattgccattgagaacgagaacctggagatcatggagctactgctgaaccacagcgtgtatgtgggtgatgcattgctctatgccatacgcaaggaagtggtgggcgctgtggagcttctgctcagctacaggcggcccagcggagagaagcaggtccccactctgatgatggacacgcagttctctgaattcacaccggacatcactcccatcatgctggctgcccacaccaacaactacgaaatcatcaaactgcttgtccaaaaacgggtcactatcccacggccccaccagatccgctgcaactgtgtggagtgtgtgtctagttcagaggtagacagcctgcgccactctcgctcccgactgaacatctataaggctctggcaagcccctcactcattgccttatcaagtgaggaccccatcctaactgccttccgtctgggctgggagctcaaggagctcagcaaggtggagaatgagttcaaggccgagtatgaggagctctctcagcagtgcaagctctttgccaaagacctgctggaccaagctcggagctccagggaactggagatcatcctcaaccatcgagatgaccacagtgaagagcttgaccctcagaagtaccatgacctggccaagttgaaggtggcaatcaaataccaccagaaagagtttgttgctcagcccaactgccaacagttgcttgccaccctgtggtatgatggcttccctggatggcggcggaaacactgggtagtcaagcttctaacctgcatgaccattgggttcctgtttcccatgctgtctatagcctacctgatctcacccaggagcaaccttgggctgttcatcaagaaaccctttatcaagtttatctgccacacagcatcctatttgaccttcctctttatgcttctcctggcttctcagcacattgtcaggacagaccttcatgtacaggggcctcccccaactgtcgtggaatggatgatattgccttgggttctaggtttcatttggggtgagattaaggaaatgtgggatggtggatttactgaatacatccatgactggtggaacctgatggattttgcaatgaactccctctacctggcaactatttccctgaagattgtggcctatgtcaagtataatggttctcgtccaagggaggaatgggaaatgtggcacccgactctgattgcggaagcactcttcgcaatatccaacattttaagttcgttgcgtctcatatccctgttcacagccaactcccacttaggacctctgcagatctctttgggacgcatgctgcttgatatcctcaaattcctctttatctactgcctggtactactagcttttgccaatggactgaaccagctttacttctattatgaaaccagagctatcgatgagcctaacaactgcaaggggatccgatgtgagaaacagaacaatgccttctccacgctctttgagactcttcagtcactcttctggtctgtatttggccttttaaatctatatgtcaccaatgtgaaagccagacacgaattcaccgagtttgtaggagctaccatgtttggaacatacaatgtcatctccctggtagtgctgctgaacatgctgattgctatgatgaacaactcctatcagcttattgccgatcatgctgatatcgagtggaagtttgcaaggacgaagctctggatgagttactttgatgaaggtggcaccttgccacctcctttcaacatcatccccagccccaagtcatttctataccttggtaactggttcaacaacaccttctgccccaaaagagaccctgacggtagacggagaaggcgcaacttgagaagtttcacagaacgcaatgctgacagcctgatacaaaatcaacattatcaggaagttatcaggaatttagtcaaaagatatgtggctgctatgataagaaattccaaaacacatgagggacttacagaagaaaattttaaggaattaaagcaagacatctccagctttcggtatgaagtgcttgacctcttgggaaatagaaaacatccaaggagcttttccactagcagcactgaactgtctcagagagacgataataatgatggcagtggtggggctcgggccaaatccaagagtgtctcttttaatttaggctgcaagaaaaagacttgccatgggccacctctcatcagaaccatgccaaggtccagtggtgcccaaggaaagtcaaaagctgagtcatcaagcaaacgctccttcatgggtccttctctcaagaaactgggtctcctattctccaaatttaatggtcatatgtctgaacccagttcagagccaatgtacacaatttctgatggaattgttcagcagcactgtatgtggcaggacatcagatattctcagatggagaaagggaaagcagaggcctgttctcaaagtgaaattaacctcagtgaggtagaattaggtgaagtccagggcgctgctcagagcagtgaatgccctctagcctgttccagctctcttcactgtgcatccagcatctgctcctcaaattctaaacttttagactcctcagaggatgtatttgaaacttggggagaggcttgtgacttgctcatgcacaaatggggtgatggacaggaagaacaagttacaactcgcctctaatgactcgagtctagagggcccgtttaaacccgctgatcagcctcgactgtgccttctagttgccagccatctgttgtttgcccctcccccgtgccttccttgaccctggaaggtgccactcccactgtcctttcctaataaaatgaggaaattgcatcgcattgtctgagtaggtgtcattctattctggggggtggggtggggcaggacagcaagggggaggattgggaagacaatagcaggcatgctggggatgcggtgggctctatggcttctgaggcggaaagaaccagctggggctctagggggtatccccacgcgccctgtagcggcgcattaagcgcggcgggtgtggtggttacgcgcagcgtgaccgctacacttgccagcgccctagcgcccgctcctttcgctttcttcccttcctttctcgccacgttcgccggctttccccgtcaagctctaaatcgggggctccctttagggttccgatttagtgctttacggcacctcgaccccaaaaaacttgattagggtgatggttcacgtagtgggccatcgccctgatagacggtttttcgccctttgacgttggagtccacgttctttaatagtggactcttgttccaaactggaacaacactcaaccctatctcggtctattcttttgatttataagggattttgccgatttcggcctattggttaaaaaatgagctgatttaacaaaaatttaacgcgaattaattctgtggaatgtgtgtcagttagggtgtggaaagtccccaggctccccagcaggcagaagtatgcaaagcatgcatctcaattagtcagcaaccaggtgtggaaagtccccaggctccccagcaggcagaagtatgcaaagcatgcatctcaattagtcagcaaccatagtcccgcccctaactccgcccatcccgcccctaactccgcccagttccgcccattctccgccccatggctgactaattttttttatttatgcagaggccgaggccgcctctgcctctgagctattccagaagtagtgaggaggcttttttggaggcctaggcttttgcaaaaagctcccgggagcttgtatatccattttcggatctgatcagcacgtgatgaaaaagcctgaactcaccgcgacgtctgtcgagaagtttctgatcgaaaagttcgacagcgtctccgacctgatgcagctctcggagggcgaagaatctcgtgctttcagcttcgatgtaggagggcgtggatatgtcctgcgggtaaatagctgcgccgatggtttctacaaagatcgttatgtttatcggcactttgcatcggccgcgctcccgattccggaagtgcttgacattggggaattcagcgagagcctgacctattgcatctcccgccgtgcacagggtgtcacgttgcaagacctgcctgaaaccgaactgcccgctgttctgcagccggtcgcggaggccatggatgcgatcgctgcggccgatcttagccagacgagcgggttcggcccattcggaccgcaaggaatcggtcaatacactacatggcgtgatttcatatgcgcgattgctgatccccatgtgtatcactggcaaactgtgatggacgacaccgtcagtgcgtccgtcgcgcaggctctcgatgagctgatgctttgggccgaggactgccccgaagtccggcacctcgtgcacgcggatttcggctccaacaatgtcctgacggacaatggccgcataacagcggtcattgactggagcgaggcgatgttcggggattcccaatacgaggtcgccaacatcttcttctggaggccgtggttggcttgtatggagcagcagacgcgctacttcgagcggaggcatccggagcttgcaggatcgccgcggctccgggcgtatatgctccgcattggtcttgaccaactctatcagagcttggttgacggcaatttcgatgatgcagcttgggcgcagggtcgatgcgacgcaatcgtccgatccggagccgggactgtcgggcgtacacaaatcgcccgcagaagcgcggccgtctggaccgatggctgtgtagaagtactcgccgatagtggaaaccgacgccccagcactcgtccgagggcaaaggaatagcacgtgctacgagatttcgattccaccgccgccttctatgaaaggttgggcttcggaatcgttttccgggacgccggctggatgatcctccagcgcggggatctcatgctggagttcttcgcccaccccaacttgtttattgcagcttataatggttacaaataaagcaatagcatcacaaatttcacaaataaagcatttttttcactgcattctagttgtggtttgtccaaactcatcaatgtatcttatcatgtctgtataccgtcgacctctagctagagcttggcgtaatcatggtcatagctgtttcctgtgtgaaattgttatccgctcacaattccacacaacatacgagccggaagcataaagtgtaaagcctggggtgcctaatgagtgagctaactcacattaattgcgttgcgctcactgcccgctttccagtcgggaaacctgtcgtgccagctgcattaatgaatcggccaacgcgcggggagaggcggtttgcgtattgggcgctcttccgcttcctcgctcactgactcgctgcgctcggtcgttcggctgcggcgagcggtatcagctcactcaaaggcggtaatacggttatccacagaatcaggggataacgcaggaaagaacatgtgagcaaaaggccagcaaaaggccaggaaccgtaaaaaggccgcgttgctggcgtttttccataggctccgcccccctgacgagcatcacaaaaatcgacgctcaagtcagaggtggcgaaacccgacaggactataaagataccaggcgtttccccctggaagctccctcgtgcgctctcctgttccgaccctgccgcttaccggatacctgtccgcctttctcccttcgggaagcgtggcgctttctcatagctcacgctgtaggtatctcagttcggtgtaggtcgttcgctccaagctgggctgtgtgcacgaaccccccgttcagcccgaccgctgcgccttatccggtaactatcgtcttgagtccaacccggtaagacacgacttatcgccactggcagcagccactggtaacaggattagcagagcgaggtatgtaggcggtgctacagagttcttgaagtggtggcctaactacggctacactagaagaacagtatttggtatctgcgctctgctgaagccagttaccttcggaaaaagagttggtagctcttgatccggcaaacaaaccaccgctggtagcggttggttttttgtttgcaagcagcagattacgcgcagaaaaaaaggatctcaagaagatcctttgatcttttctacggggtctgacgctcagtggaacgaaaactcacgttaagggattttggtcatgagattatcaaaaaggatcttcacctagatccttttaaattaaaaatgaagttttaaatcaatctaaagtatatatgagtaaacttggtctgacagttaccaatgcttaatcagtgaggcacctatctcagcgatctgtctatttcgttcatccatagttgcctgactccccgtcgtgtagataactacgatacgggagggcttaccatctggccccagtgctgcaatgataccgcgagacccacgctcaccggctccagatttatcagcaataaaccagccagccggaagggccgagcgcagaagtggtcctgcaactttatccgcctccatccagtctattaattgttgccgggaagctagagtaagtagttcgccagttaatagtttgcgcaacgttgttgccattgctacaggcatcgtggtgtcacgctcgtcgtttggtatggcttcattcagctccggttcccaacgatcaaggcgagttacatgatcccccatgttgtgcaaaaaagcggttagctccttcggtcctccgatcgttgtcagaagtaagttggccgcagtgttatcactcatggttatggcagcactgcataattctcttactgtcatgccatccgtaagatgcttttctgtgactggtgagtactcaaccaagtcattctgagaatagtgtatgcggcgaccgagttgctcttgcccggcgtcaatacgggataataccgcgccacatagcagaactttaaaagtgctcatcattggaaaacgttcttcggggcgaaaactctcaaggatcttaccgctgttgagatccagttcgatgtaacccactcgtgcacccaactgatcttcagcatcttttactttcaccagcgtttctgggtgagcaaaaacaggaaggcaaaatgccgcaaaaaagggaataagggcgacacggaaatgttgaatactcatactcttcctttttcaatattattgaagcatttatcagggttattgtctcatgagcggatacatatttgaatgtatttagaaaaataaacaaataggggttccgcgcacatttccccgaaaagtgccacctgacgtc